European Patent Application EP 4 438 617 A1, published October 2, 2024. Title: Peptides having inhibitory activity against amyloid precursor protein and uses thereof. Applicant: WINGSTABIO INC. The sequence listing filed with the application follows.

SEQUENCE LISTING (25 sequences)

SEQ ID NO: 1 - protein, 14 aa, synthetic construct
LKLKALAALIKKIL

SEQ ID NO: 2 - protein, 14 aa, synthetic construct
IKLLSIVAWAKKKI

SEQ ID NO: 3 - protein, 13 aa, synthetic construct
INLKALAAKIKIL

SEQ ID NO: 4 - protein, 12 aa, synthetic construct
INIKVLIAKKIL

SEQ ID NO: 5 - protein, 12 aa, synthetic construct
LNIRGLGAKKKI

SEQ ID NO: 6 - protein, 11 aa, synthetic construct
LNLRGLAKKKL

SEQ ID NO: 7 - protein, 11 aa, synthetic construct
KALAALAKKIL

SEQ ID NO: 8 - protein, 9 aa, synthetic construct
KALAALAKK

SEQ ID NO: 9 - protein, 14 aa, synthetic construct
AFMVDNEAIYDICR

SEQ ID NO: 10 - DNA, 20 bp, synthetic construct
  source 1..20: mol_type = other DNA
ccgaggggtagagtttgtgt

SEQ ID NO: 11 - DNA, 20 bp, synthetic construct
  source 1..20: mol_type = other DNA
acctcagccacttcttcctc

SEQ ID NO: 12 - DNA, 21 bp, synthetic construct
  source 1..21: mol_type = other DNA
accacagacttctccggaatc

SEQ ID NO: 13 - DNA, 21 bp, synthetic construct
  source 1..21: mol_type = other DNA
ggtctgtgaagacataggcca

SEQ ID NO: 14 - DNA, 19 bp, synthetic construct
  source 1..19: mol_type = other DNA
tcgcttctacagcatgggc

SEQ ID NO: 15 - DNA, 20 bp, synthetic construct
  source 1..20: mol_type = other DNA
tgagaatgcgaatctgctct

SEQ ID NO: 16 - DNA, 20 bp, synthetic construct
  source 1..20: mol_type = other DNA
aaagaggcgagaccataccc

SEQ ID NO: 17 - DNA, 20 bp, synthetic construct
  source 1..20: mol_type = other DNA
gcaaggggtccacataagca

SEQ ID NO: 18 - DNA, 17 bp, synthetic construct
  source 1..17: mol_type = other DNA
ccccaagctgagaacca

SEQ ID NO: 19 - DNA, 20 bp, synthetic construct
  source 1..20: mol_type = other DNA
tctcaaggggctgggtcagc

SEQ ID NO: 20 - protein, 14 aa, synthetic construct
INLLKIAGKIINIL

SEQ ID NO: 21 - protein, 14 aa, synthetic construct
INLLKSEGKIIKSL

SEQ ID NO: 22 - protein, 10 aa, synthetic construct
GRPPGFSLAR

SEQ ID NO: 23 - protein, 10 aa, synthetic construct
GRILGFSPFR

SEQ ID NO: 24 - DNA, 20 bp, synthetic construct
  source 1..20: mol_type = other DNA
ggcggcagacaaaaagactg

SEQ ID NO: 25 - DNA, 20 bp, synthetic construct
  source 1..20: mol_type = other DNA
cactgggagttccaatgcct